European Patent Specification EP 3 368 654 B1, published November 19, 2025. Title: DETERMINATION OF POLYMORPHISMS USING ISOTHERMAL NUCLEIC ACID AMPLIFICATION. Applicant: Alere Inc. The sequence listing filed with the application follows.

SEQUENCE LISTING (15 sequences)

SEQ ID NO: 1 - DNA, 49 bp, Homo sapiens
atctgactcctgaggagaagtctgccgttactgccctgtggggcaaggt

SEQ ID NO: 2 - DNA, 49 bp, Homo sapiens
atctgactcctgtggagaagtctgccgttactgccctgtggggcaaggt

SEQ ID NO: 3 - DNA, 49 bp, Homo sapiens
atctgactcctgtggacaagtctgccgttactgccctgtggggcaaggt

SEQ ID NO: 4 - DNA, 49 bp, Homo sapiens
atctgactcctgaggacaagtctgccgttactgccctgtggggcaaggt

SEQ ID NO: 5 - DNA, 32 bp, Artificial Sequence
  synthetic primer
catctattgcttacatttgcttctgacacaac

SEQ ID NO: 6 - DNA, 35 bp, Artificial Sequence
  synthetic primer
accttgccccacagggcagtaacggcagacttgtc

SEQ ID NO: 7 - DNA, 45 bp, Artificial Sequence
  synthetic probe
  misc_feature (30)..(31): T at residue 30 and G at residue 31 can be separated by a spacer
  misc_feature (30)..(30): T at residue 30 is conjugated to a ROX fluorescent dye
  misc_feature (32)..(32): BHQ-2 fluorescent quencher
  misc_feature (44)..(45): C at residue 44 and T at residue 45 are connected by a phosphothioate bond
tgttcactagcaacctcaaacagacaccatgtgcatctgactcct

SEQ ID NO: 8 - DNA, 278 bp, Homo sapiens
gagcagagtcagaatccttcagaaggctttttctttagacagttgtttgttcagttgggagcggagccacgtgttgaagtcctcgttgtcttgttggcaggggtctgcacccgggagcccccgttctatatcatcactgagttcatgacctacgggaacctcctggactacctgagggagtgcaaccggcaggaggtgaacgccgtggtgctgctgtacatggccactcagatctcgtcagccatggagtacctggagaagaaaaacttcatccacag

SEQ ID NO: 9 - DNA, 224 bp, Homo sapiens
  misc_feature (151)..(151): n is a, c, g, or t
gttggccaatctactcccaggagcagggagggcaggagccagggctgggcataaaagtcagggcagagccatctattgcttacatttgcttctgacacaactgtgttcactagcaacctcaaacagacaccatggtgcatctgactcctgnggagaagtctgccgttactgccctgtggggcaaggtgaacgtggatgaagttggtggtgaggccctgggcagg

SEQ ID NO: 10 - DNA, 18 bp, Artificial Sequence
  synthetic primer
actgaggactcctcttca

SEQ ID NO: 11 - DNA, 18 bp, Artificial Sequence
  synthetic primer
tgactcctgaggagaagt

SEQ ID NO: 12 - DNA, 18 bp, Artificial Sequence
  synthetic primer
tgactcctgtggagaagt

SEQ ID NO: 13 - DNA, 18 bp, Artificial Sequence
  synthetic primer
actgaggacacctcttca

SEQ ID NO: 14 - DNA, 18 bp, Artificial Sequence
  synthetic primer
tgactcctgaggagaagt

SEQ ID NO: 15 - DNA, 18 bp, Artificial Sequence
  synthetic primer
tgactcctgtggagaagt